European Patent Application EP 4 483 897 A1, published January 1, 2025. Title: SZCZEPIONKA I PREPARAT UODPARNIAJĄCY I/LUB LECZNICZY DO STOSOWANIA W ZAPOBIEGANIU I/LUB LECZENIU KOLIBAKTERIOZ U PROSIĄT. Applicant: Zakład Badawczo-Wdrożeniowy Ośrodka Salmonella "IMMUNOLAB" Sp. z o. o. The sequence listing filed with the application follows.

SEQUENCE LISTING (6 sequences)

SEQ ID NO: 1 - protein, 68 aa, E. coli
ADCAKGKIEFSKYNEDNTFTVKVSGREYWTNRWNLQPLLQSAQLTGMTVTIISNTCSSGSGFAQVKFN

SEQ ID NO: 2 - DNA, 207 bp, E. coli
  source 1..207: mol_type = unassigned DNA
gcggattgtgctaaaggtaaaattgagttttccaagtataatgaggataatacctttactgtgaaggtgtcaggaagagaatactggacgaacagatggaatttgcagccattgttacaaagtgctcagctgacagggatgactgtaacaatcatatctaatacctgcagttcaggctcaggctttgcccaggtgaagtttaactga

SEQ ID NO: 3 - protein, 74 aa, E. coli
HHHHHHADCAKGKIEFSKYNEDNTFTVKVSGREYWTNRWNLQPLLQSAQLTGMTVTIISNTCSSGSGFAQVKFN

SEQ ID NO: 4 - DNA, 228 bp, E. coli
  source 1..228: mol_type = unassigned DNA
atgcaccaccatcatcaccacgcggattgtgctaaaggtaaaattgagttttccaagtataatgaggataatacctttactgtgaaggtgtcaggaagagaatactggacgaacagatggaatttgcagccattgttacaaagtgctcagctgacagggatgactgtaacaatcatatctaatacctgcagttcaggctcaggctttgcccaggtgaagtttaactga

SEQ ID NO: 5 - protein, 75 aa, E. coli
MADCAKGKIEFSKYNEDNTFTVKVSGREYWTNRWNLQPLLQSAQLTGMTVTIISNTCSSGSGFAQVKFNHHHHHH

SEQ ID NO: 6 - DNA, 228 bp, E. coli
  source 1..228: mol_type = unassigned DNA
atggcggattgtgctaaaggtaaaattgagttttccaagtataatgaggataatacctttactgtgaaggtgtcaggaagagaatactggacgaacagatggaatttgcagccattgttacaaagtgctcagctgacagggatgactgtaacaatcatatctaatacctgcagttcaggctcaggctttgcccaggtgaagtttaaccaccaccatcatcaccactga